European Patent Application EP 4 324 853 A1, published February 21, 2024. Title: MULTI-SPECIFIC ANTIBODY TARGETING BCMA. Applicant: CHIA TAI TIANQING PHARMACEUTICAL GROUP CO., LTD. Application EP22787602.6. The sequence listing filed with the application follows.

SEQUENCE LISTING (84 sequences)

SEQ ID NO: 1 - protein, 5 aa, Artificial Sequence
  Peptide linker
GGGGS

SEQ ID NO: 2 - protein, 14 aa, Artificial Sequence
  Peptide linker
GGSGGSGGSGGSGG

SEQ ID NO: 3 - protein, 16 aa, Artificial Sequence
  Hinge region
GEPKSSDKTHTCPPCP

SEQ ID NO: 4 - protein, 15 aa, Artificial Sequence
  Hinge region
EPKSCDKTHTCPPCP

SEQ ID NO: 5 - protein, 232 aa, Homo sapiens
  Human IgG1 constant region
EPKSCDKTHTCPPCPAPELLGGPSVFLFPPKPKDTLMISRTPEVTCVVVDVSHEDPEVKFNWYVDGVEVHNAKTKPREEQYNSTYRVVSVLTVLHQDWLNGKEYKCKVSNKALPAPIEKTISKAKGQPREPQVYTLPPSRDELTKNQVSLTCLVKGFYPSDIAVEWESNGQPENNYKTTPPVLDSDGSFFLYSKLTVDKSRWQQGNVFSCSVMHEALHNHYTQKSLSLSPGK

SEQ ID NO: 6 - protein, 183 aa, Macaca fascicularis
  Full-length cynomolgus monkey BCMA
MLQMARQCSQNEYFDSLLHDCKPCQLRCSSTPPLTCQRYCNASMTNSVKGMNAILWTCLGLSLIISLAVFVLTFLLRKMSSEPLKDEFKNTGSGLLGMANIDLEKGRTGDEIVLPRGLEYTVEECTCEDCIKNKPKVDSDHCFPLPAMEEGATILVTTKTNDYCNSLSAALSVTEIEKSISAR

SEQ ID NO: 7 - protein, 5 aa, Camelus bactrianus
  1A1 single variable domain CDR1
GWNKH

SEQ ID NO: 8 - protein, 16 aa, Camelus bactrianus
  1A1 single variable domain CDR2
SIFRDGKTAYTDSVKG

SEQ ID NO: 9 - protein, 10 aa, Camelus bactrianus
  1A1 single variable domain CDR3
DLPGSGLPAF

SEQ ID NO: 10 - protein, 5 aa, Camelus bactrianus
  1A10 single variable domain CDR1
VACMA

SEQ ID NO: 11 - protein, 17 aa, Camelus bactrianus
  1A10 single variable domain CDR2
TIVADFGTTNYAASVKG

SEQ ID NO: 12 - protein, 14 aa, Camelus bactrianus
  1A10 single variable domain CDR3
TQRGGIDWCDEINY

SEQ ID NO: 13 - protein, 5 aa, Camelus bactrianus
  1A11 single variable domain CDR1
SACMG

SEQ ID NO: 14 - protein, 17 aa, Camelus bactrianus
  1A11 single variable domain CDR2
RIETGYGGTVYADSVKG

SEQ ID NO: 15 - protein, 17 aa, Camelus bactrianus
  1A11 single variable domain CDR3
KRSWCTPTWWHELDYNY

SEQ ID NO: 16 - protein, 5 aa, Camelus bactrianus
  1B10 single variable domain CDR1
GWNKH

SEQ ID NO: 17 - protein, 16 aa, Camelus bactrianus
  1B10 single variable domain CDR2
SIFRDGKTAYTDSVKG

SEQ ID NO: 18 - protein, 10 aa, Camelus bactrianus
  1B10 single variable domain CDR3
DLPGSGLPEF

SEQ ID NO: 19 - protein, 118 aa, Camelus bactrianus
  1A1 single variable domain
QVQLVESGGGSVQAGGSLRLSCTASGYTFRGWNKHWYRQAPGKERELVSSIFRDGKTAYTDSVKGRFTISQDNADATVYLQMNSLKPEDTAMYYCKYDLPGSGLPAFWGQGTLVTVSS

SEQ ID NO: 20 - DNA, 354 bp, Camelus bactrianus
  1A1 single variable domain
caggtgcagctggtggagtctgggggaggctcggtgcaggccggagggtctctgagactctcctgtacagcctctggatacaccttcaggggctggaacaagcactggtaccgccaggctccagggaaggagcgcgagttggtctcgagcatctttcgtgatgggaagacagcctatacagactccgtgaagggccgattcaccatctctcaagacaacgccgacgcaacggtgtatctgcaaatgaacagcctgaaacctgaggacacggccatgtattactgtaaatacgatctgcctggatctggtcttcctgcattctggggccaggggaccctggtcactgtctcatca

SEQ ID NO: 21 - protein, 123 aa, Camelus bactrianus
  1A10 single variable domain
QVQLVESGGGSVQAGGSLRLSCAASGYSSNVACMAWYRQAPGKEREWVATIVADFGTTNYAASVKGRFTISQDNAKNTVYLQMNSLKPEDSAMYYCAATQRGGIDWCDEINYWGQGTLVTVSS

SEQ ID NO: 22 - DNA, 369 bp, Camelus bactrianus
  1A10 single variable domain
caggtgcagctggtggagtctgggggaggctcggtgcaggctggagggtcgctgagactctcctgtgccgcctccggatacagcagtaatgtggcatgcatggcctggtaccgccaggctccagggaaggagcgcgagtgggtcgcaactattgttgctgatttcggtaccacaaactatgccgcctccgtgaagggccgattcaccatctcccaagacaacgccaagaacacggtgtatctgcaaatgaacagcctgaaacctgaggactctgccatgtactactgtgcggcaacccagagggggggtattgactggtgtgatgaaattaattactggggccaggggaccctggtcactgtctcatca

SEQ ID NO: 23 - protein, 126 aa, Camelus bactrianus
  1A11 single variable domain
QVQLVESGGGSVQAGGSLRLSCAASGVTFNSACMGWFRQAPGKEREGVARIETGYGGTVYADSVKGRFTISRDNAKNTVYLQMNSLKPEDTAMYYCAAKRSWCTPTWWHELDYNYWGQGTQVTVSS

SEQ ID NO: 24 - DNA, 378 bp, Camelus bactrianus
  1A11 single variable domain
caggtgcagctggtggagtctgggggaggctcggtgcaggctggagggtctctgagactctcctgtgcagcctctggagtcacttttaatagcgcatgtatgggttggttccgccaggctccagggaaggagcgcgagggggtcgcacgtattgaaactggttatggtggcactgtctatgccgactccgtgaagggacgattcaccatctcccgagacaacgccaagaacacggtgtatctgcaaatgaacagcctaaaacctgaggacactgccatgtactactgtgcggctaagagatcctggtgtactcctacgtggtggcacgaacttgactataactactggggacaggggacccaggtcactgtctcatca

SEQ ID NO: 25 - protein, 118 aa, Camelus bactrianus
  1B10 single variable domain
EVQLVESGGGSVQAGGSLRLSCTASGYTFRGWNKHWYRQAPGKERELVSSIFRDGKTAYTDSVKGRFTISQDSADATVYLQMNSLKPEDTAMYYCKYDLPGSGLPEFWGQGTLVTVSS

SEQ ID NO: 26 - DNA, 354 bp, Camelus bactrianus
  1B10 single variable domain
gaggtgcagctggtggagtctgggggaggctcggtgcaggccggagggtctctgagactctcctgtacagcctctggatacaccttcaggggctggaacaagcactggtaccgccaggctccagggaaggagcgcgagttggtctcgagtatctttcgtgatgggaagacagcctatacagactccgtgaagggccgattcaccatctctcaagacagcgccgacgcaacggtgtatctgcaaatgaacagcctgaaacctgaggacacggccatgtattactgtaaatacgatctgcctggatctggtcttcctgagttctggggccaggggaccctggtcactgtctcatca

SEQ ID NO: 27 - protein, 350 aa, Artificial Sequence
  1A1-Fc
QVQLVESGGGSVQAGGSLRLSCTASGYTFRGWNKHWYRQAPGKERELVSSIFRDGKTAYTDSVKGRFTISQDNADATVYLQMNSLKPEDTAMYYCKYDLPGSGLPAFWGQGTLVTVSSEPKSCDKTHTCPPCPAPELLGGPSVFLFPPKPKDTLMISRTPEVTCVVVDVSHEDPEVKFNWYVDGVEVHNAKTKPREEQYNSTYRVVSVLTVLHQDWLNGKEYKCKVSNKALPAPIEKTISKAKGQPREPQVYTLPPSRDELTKNQVSLTCLVKGFYPSDIAVEWESNGQPENNYKTTPPVLDSDGSFFLYSKLTVDKSRWQQGNVFSCSVMHEALHNHYTQKSLSLSPGK

SEQ ID NO: 28 - DNA, 1050 bp, Artificial Sequence
  1A1-Fc
caagtgcaactggtggagtctggaggcggttccgtgcaggccggcggctccctgagactgtcctgcaccgcttccggctacaccttcagaggctggaacaagcactggtatcggcaggctcctggcaaagaaagagagctggtgtcctccatcttccgggacggcaagaccgcctacaccgactccgtgaagggcagattcaccatctctcaggacaacgccgacgccacagtgtacctgcagatgaactctctgaagcccgaggacaccgccatgtactactgcaagtacgacctgcctggatctggcctgcccgccttctggggccaaggcaccctggtaaccgtgtcgtccgagcccaagtcttgcgacaagacccacacctgtcctccttgtcctgctccggaactgctgggcggcccttccgtgtttctgtttcctccaaagcctaaggacacactgatgatcagccggacccctgaggtgacctgcgtggtcgtggatgtctctcacgaggatcctgaggtgaagttcaactggtacgtggatggagtggaagtgcataacgctaaaaccaagcctagagaagagcagtacaactccacctacagagtggtgtccgtgctgaccgtgctgcaccaggattggctgaacggcaaagagtacaagtgcaaggtgtccaacaaggctctgcctgcccctatcgagaagaccatctccaaggccaagggccagcctcgggagcctcaagtgtacaccctgcctccttctcgcgacgagctgaccaagaaccaggtgtctctgacctgcctggtgaaaggcttctacccctccgacatcgccgtggaatgggagtccaatggccagcccgagaacaactacaagaccaccccacctgtgctggactctgatggctccttcttcctgtactccaagctgaccgtggacaagtccagatggcagcagggcaacgtgttctcctgttctgtgatgcacgaggccctgcacaaccactacacacagaagtccctgagcctgtctcctggcaag

SEQ ID NO: 29 - protein, 355 aa, Artificial Sequence
  1A10-Fc
QVQLVESGGGSVQAGGSLRLSCAASGYSSNVACMAWYRQAPGKEREWVATIVADFGTTNYAASVKGRFTISQDNAKNTVYLQMNSLKPEDSAMYYCAATQRGGIDWCDEINYWGQGTLVTVSSEPKSCDKTHTCPPCPAPELLGGPSVFLFPPKPKDTLMISRTPEVTCVVVDVSHEDPEVKFNWYVDGVEVHNAKTKPREEQYNSTYRVVSVLTVLHQDWLNGKEYKCKVSNKALPAPIEKTISKAKGQPREPQVYTLPPSRDELTKNQVSLTCLVKGFYPSDIAVEWESNGQPENNYKTTPPVLDSDGSFFLYSKLTVDKSRWQQGNVFSCSVMHEALHNHYTQKSLSLSPGK

SEQ ID NO: 30 - DNA, 1065 bp, Artificial Sequence
  1A10-Fc
caggtgcaactggtggagtctggcggcggatctgtgcaagctggcggatccctgagactgtcttgtgccgcttccggctactcctctaacgtggcctgtatggcctggtacagacaggcccctggcaaagaaagagagtgggtcgccaccatcgtggccgatttcggcaccaccaattacgccgcttccgtgaagggcagattcaccatctctcaggacaacgccaagaacaccgtgtacctgcagatgaactccctgaagcctgaggactccgccatgtactactgcgccgctacacagcgcggaggcattgattggtgcgacgagattaactactggggccaaggcaccctggttaccgtgtcctctgagcccaagtcctgcgacaagacccacacctgtccaccttgtcctgccccagaactgctgggcggtcccagcgtgttcctgttcccccccaagcctaaggacacactgatgatctctagaacccctgaagtgacctgcgtggtggtcgatgtatctcacgaggatcctgaggtcaagttcaactggtacgtggacggagtggaagtgcataatgctaagaccaagcctagagaggaacagtacaactccacctacagagtggtgtccgtgctgaccgtgctgcaccaggattggctgaacggcaaggagtacaagtgcaaggtgtccaacaaggctctgcctgctcctatcgagaagaccatcagcaaggccaagggccagcctcgggagcctcaagtgtacaccctgcctccttctcgggacgagctgaccaagaaccaggtgtctcttacatgcctggtgaaaggcttctacccttccgacatcgccgtggaatgggagtccaatggccagcccgagaacaactacaagaccacacctcctgtgctggactctgacggctccttcttcctgtactccaagctgacagtggataagtccagatggcagcagggcaacgtgttctcctgctccgtgatgcacgaggccctgcacaaccactacacccagaagtctctgagcctgtcccctggaaaa

SEQ ID NO: 31 - protein, 358 aa, Artificial Sequence
  1A11-Fc
QVQLVESGGGSVQAGGSLRLSCAASGVTFNSACMGWFRQAPGKEREGVARIETGYGGTVYADSVKGRFTISRDNAKNTVYLQMNSLKPEDTAMYYCAAKRSWCTPTWWHELDYNYWGQGTQVTVSSEPKSCDKTHTCPPCPAPELLGGPSVFLFPPKPKDTLMISRTPEVTCVVVDVSHEDPEVKFNWYVDGVEVHNAKTKPREEQYNSTYRVVSVLTVLHQDWLNGKEYKCKVSNKALPAPIEKTISKAKGQPREPQVYTLPPSRDELTKNQVSLTCLVKGFYPSDIAVEWESNGQPENNYKTTPPVLDSDGSFFLYSKLTVDKSRWQQGNVFSCSVMHEALHNHYTQKSLSLSPGK

SEQ ID NO: 32 - DNA, 1074 bp, Artificial Sequence
  1A11-Fc
caggtgcagttggttgaatctggcggcggatctgtgcaggctggcggatctctgagactgtcctgtgccgcttccggcgtcaccttcaactccgcttgcatgggatggttcagacaggcccctggcaaagagagagagggcgtcgctaggatcgagaccggctatggcggaaccgtctacgccgactccgtcaagggcaggttcaccatcagcagagacaacgccaagaacaccgtgtacctgcagatgaactccctgaagcccgaggacaccgccatgtactactgtgctgccaagagaagctggtgcacccctacctggtggcacgagctggactacaactactggggccagggcacacaggtcaccgtgtcctctgagcctaagtcctgcgacaagacccacacctgtcctccatgtcctgctccagaactgctcggcggaccttccgtgttcctgtttcctccaaagcctaaggataccctgatgatctctcggacccctgaagtgacctgcgtggtggtggatgtgtctcacgaggatcccgaagtgaagttcaattggtacgtggacggcgtggaagtgcacaatgctaagaccaagcctagagaggaacagtacaactccacctatagagtggtgtccgtgctgaccgtgctgcaccaggattggctgaacggcaaagagtacaagtgcaaggtgtccaacaaggccctgcctgctcctatcgaaaagaccatctccaaggccaagggccagcctagggaaccccaggtttacaccttgcctccatctcgggacgagctgaccaagaaccaggtgtccctgacctgtctggtcaagggcttctacccctccgatatcgccgtggaatgggagtctaatggccagccagagaacaactacaagacaacccctcctgtgctggactccgacggctcattcttcctgtactccaagctgacagtggacaagtccagatggcagcagggcaacgtgttctcctgctccgtgatgcacgaggccctgcacaatcactacacccagaagtccctgtctctgagccccggcaaa

SEQ ID NO: 33 - protein, 350 aa, Artificial Sequence
  1B10-Fc
EVQLVESGGGSVQAGGSLRLSCTASGYTFRGWNKHWYRQAPGKERELVSSIFRDGKTAYTDSVKGRFTISQDSADATVYLQMNSLKPEDTAMYYCKYDLPGSGLPEFWGQGTLVTVSSEPKSCDKTHTCPPCPAPELLGGPSVFLFPPKPKDTLMISRTPEVTCVVVDVSHEDPEVKFNWYVDGVEVHNAKTKPREEQYNSTYRVVSVLTVLHQDWLNGKEYKCKVSNKALPAPIEKTISKAKGQPREPQVYTLPPSRDELTKNQVSLTCLVKGFYPSDIAVEWESNGQPENNYKTTPPVLDSDGSFFLYSKLTVDKSRWQQGNVFSCSVMHEALHNHYTQKSLSLSPGK

SEQ ID NO: 34 - DNA, 1050 bp, Artificial Sequence
  1B10-Fc
gaggtgcaactggtggagtctggaggcggttccgtgcaggccggcggctccctgagactgtcctgcaccgcttccggctacaccttcagaggctggaacaagcactggtatcggcaggctcctggcaaagaaagagagctggtgtcctccatcttccgggacggcaagaccgcctacaccgactccgtgaagggcagattcaccatctctcaggactctgccgacgccacagtgtacctgcagatgaactctctgaagcccgaggacaccgccatgtactactgcaagtacgacctgcctggatctggcctgcccgagttctggggccaaggcaccctggtaaccgtgtcgtccgagcccaagtcttgcgacaagacccacacctgtcctccttgtcctgctccggaactgctgggcggcccttccgtgtttctgtttcctccaaagcctaaggacacactgatgatcagccggacccctgaggtgacctgcgtggtcgtggatgtctctcacgaggatcctgaggtgaagttcaactggtacgtggatggagtggaagtgcataacgctaaaaccaagcctagagaagagcagtacaactccacctacagagtggtgtccgtgctgaccgtgctgcaccaggattggctgaacggcaaagagtacaagtgcaaggtgtccaacaaggctctgcctgcccctatcgagaagaccatctccaaggccaagggccagcctcgggagcctcaagtgtacaccctgcctccttctcgcgacgagctgaccaagaaccaggtgtctctgacctgcctggtgaaaggcttctacccctccgacatcgccgtggaatgggagtccaatggccagcccgagaacaactacaagaccaccccacctgtgctggactctgatggctccttcttcctgtactccaagctgaccgtggacaagtccagatggcagcagggcaacgtgttctcctgttctgtgatgcacgaggccctgcacaaccactacacacagaagtccctgagcctgtctcctggcaag

SEQ ID NO: 35 - protein, 54 aa, Homo sapiens
  Human BCMA extracellular region
MLQMAGQCSQNEYFDSLLHACIPCQLRCSSNTPPLTCQRYCNASVTNSVKGTNA

SEQ ID NO: 36 - protein, 53 aa, Macaca fascicularis
  Cynomolgus monkey BCMA extracellular region
MLQMARQCSQNEYFDSLLHDCKPCQLRCSSTPPLTCQRYCNASMTNSVKGMNA

SEQ ID NO: 37 - protein, 123 aa, Artificial Sequence
  1A10-V1 single variable domain
QVQLVESGGGLVQPGGSLRLSCAASGYSSNVACMAWYRQAPGKGLEWVATIVADFGTTNYAASVKGRFTISQDNSKNTVYLQMNSLRAEDTAVYYCAATQRGGIDWCDEINYWGQGTLVTVSS

SEQ ID NO: 38 - protein, 123 aa, Artificial Sequence
  1A10-V2 single variable domain
QVQLVESGGGLVQPGGSLRLSCAASGYSSNVACMAWYRQAPGKEREWVSTIVADFGTTNYAASVKGRFTISQDNSKNTVYLQMNSLRAEDTAVYYCAATQRGGIDWCDEINYWGQGTLVTVSS

SEQ ID NO: 39 - protein, 126 aa, Artificial Sequence
  1A11-V1 single variable domain
QVQLVESGGGLVQPGGSLRLSCAASGFTFNSACMGWFRQAPGKGREGVSRIETGYGGTVYADSVKGRFTISRDNSKNTVYLQMNSLRAEDTAVYYCAAKRSWCTPTWWHELDYNYWGQGTQVTVSS

SEQ ID NO: 40 - protein, 126 aa, Artificial Sequence
  1A11-V2 single variable domain
QVQLVESGGGLVQPGGSLRLSCAASGFTFNSACMGWFRQAPGKEREGVSRIETGYGGTVYADSVKGRFTISRDNSKNTVYLQMNSLKAEDTAVYYCAAKRSWCTPTWWHELDYNYWGQGTQVTVSS

SEQ ID NO: 41 - protein, 123 aa, Artificial Sequence
  UNSURE (11): Xaa is S or L
  UNSURE (14): Xaa is P or A
  UNSURE (44): Xaa is G or E
  UNSURE (45): Xaa is R or L
  UNSURE (49): Xaa is A or S
  UNSURE (75): Xaa is A or S
  UNSURE (87): Xaa is R or K
  UNSURE (88): Xaa is A or P
  UNSURE (91): Xaa is T or S
  UNSURE (93): Xaa is V or M
  BCMA-binding single variable domain
QVQLVESGGGXVQXGGSLRLSCAASGYSSNVACMAWYRQAPGKXXEWVXTIVADFGTTNYAASVKGRFTISQDNXKNTVYLQMNSLXXEDXAXYYCAATQRGGIDWCDEINYWGQGTLVTVSS

SEQ ID NO: 42 - protein, 126 aa, Artificial Sequence
  UNSURE (11): Xaa is S or L
  UNSURE (14): Xaa is P or A
  UNSURE (27): Xaa is F or V
  UNSURE (44): Xaa is E or G
  UNSURE (49): Xaa is A or S
  UNSURE (75): Xaa is A or S
  UNSURE (87): Xaa is R or K
  UNSURE (88): Xaa is A or P
  UNSURE (93): Xaa is V or M
  BCMA-binding single variable domain
QVQLVESGGGXVQXGGSLRLSCAASGXTFNSACMGWFRQAPGKXREGVXRIETGYGGTVYADSVKGRFTISRDNXKNTVYLQMNSLXXEDTAXYYCAAKRSWCTPTWWHELDYNYWGQGTQVTVSS

SEQ ID NO: 43 - protein, 5 aa, Artificial Sequence
  CD3-HCDR1
TYAMN

SEQ ID NO: 44 - protein, 19 aa, Artificial Sequence
  CD3-HCDR2
RIRSKYNNYATYYADSVKD

SEQ ID NO: 45 - protein, 14 aa, Artificial Sequence
  CD3-HCDR3
HGNFGNSYVSWFAY

SEQ ID NO: 46 - protein, 14 aa, Artificial Sequence
  CD3-LCDR1
RSSTGAVTTSNYAN

SEQ ID NO: 47 - protein, 7 aa, Artificial Sequence
  CD3-LCDR2
GTNKRAP

SEQ ID NO: 48 - protein, 9 aa, Artificial Sequence
  CD3-LCDR3
ALWYSNLWV

SEQ ID NO: 49 - protein, 125 aa, Artificial Sequence
  CD3-VH
EVQLVESGGGLVQPGGSLRLSCAASGFTFNTYAMNWVRQAPGKGLEWVARIRSKYNNYATYYADSVKDRFTISRDDSKNTAYLQMNNLKTEDTAMYYCVRHGNFGNSYVSWFAYWGQGTLVTVSS

SEQ ID NO: 50 - protein, 109 aa, Artificial Sequence
  CD3-VL
ELVVTQEPSLTTSPGGTVTLTCRSSTGAVTTSNYANWVQQKPGQAPRGLIGGTNKRAPGTPARFSGSLLGGKAALTITGVQPEDEAEYYCALWYSNLWVFGGGTKLTVL

SEQ ID NO: 51 - protein, 356 aa, Artificial Sequence
  1A10-V1
QVQLVESGGGLVQPGGSLRLSCAASGYSSNVACMAWYRQAPGKGLEWVATIVADFGTTNYAASVKGRFTISQDNSKNTVYLQMNSLRAEDTAVYYCAATQRGGIDWCDEINYWGQGTLVTVSSGEPKSSDKTHTCPPCPAPELLGGPSVFLFPPKPKDTLMISRTPEVTCVVVDVSHEDPEVKFNWYVDGVEVHNAKTKPREEQYNSTYRVVSVLTVLHQDWLNGKEYKCKVSNKALPAPIEKTISKAKGQPREPQVYTLPPSRDELTKNQVSLTCLVKGFYPSDIAVEWESNGQPENNYKTTPPVLDSDGSFFLYSKLTVDKSRWQQGNVFSCSVMHEALHNHYTQKSLSLSPGK

SEQ ID NO: 52 - DNA, 1068 bp, Artificial Sequence
  1A10-V1
caggtgcagctggtggagtccggcggcggactggtgcagcctggaggatctctgcggctgtcctgcgccgccagcggatactccagcaacgtggcttgcatggcctggtatcggcaggcccctggcaagggcctggagtgggtggctaccatcgtggctgacttcggcaccaccaattatgccgctagcgtgaagggccggttcaccatcagccaggataactccaagaataccgtgtatctgcagatgaatagcctgcgggccgaggataccgccgtgtattattgtgccgctacccagcggggcggcatcgactggtgtgatgagatcaactattggggccagggcaccctggtgaccgtgtcctccggcgagcctaagtcctccgacaagacccacacctgccctccttgtcccgcccctgagctgctgggcggaccatctgtgttcctgttccctcccaagcccaaggacaccctgatgatctccaggacccctgaggtgacctgcgtggtggtggatgtgtcccacgaggaccctgaggtgaagttcaactggtacgtggacggcgtggaggtgcacaatgctaagaccaagccccgggaggagcagtataacagcacctaccgggtggtgagcgtgctgaccgtgctgcaccaggattggctgaatggcaaggagtacaagtgtaaggtgtccaacaaggctctgcctgcccccatcgagaagaccatctccaaggccaagggccagcctcgggagccccaggtgtataccctgcccccctccagggacgagctgaccaagaaccaggtgagcctgacctgtctggtgaagggcttctatccttccgacatcgccgtggagtgggagtccaacggccagcctgagaataactacaagaccaccccccctgtgctggatagcgacggctccttcttcctgtattccaagctgaccgtggataagtcccggtggcagcagggcaatgtgttcagctgttccgtgatgcacgaggctctgcacaaccactatacccagaagtccctgtccctgagccccggcaag

SEQ ID NO: 53 - protein, 356 aa, Artificial Sequence
  1A10-V2
QVQLVESGGGLVQPGGSLRLSCAASGYSSNVACMAWYRQAPGKEREWVSTIVADFGTTNYAASVKGRFTISQDNSKNTVYLQMNSLRAEDTAVYYCAATQRGGIDWCDEINYWGQGTLVTVSSGEPKSSDKTHTCPPCPAPELLGGPSVFLFPPKPKDTLMISRTPEVTCVVVDVSHEDPEVKFNWYVDGVEVHNAKTKPREEQYNSTYRVVSVLTVLHQDWLNGKEYKCKVSNKALPAPIEKTISKAKGQPREPQVYTLPPSRDELTKNQVSLTCLVKGFYPSDIAVEWESNGQPENNYKTTPPVLDSDGSFFLYSKLTVDKSRWQQGNVFSCSVMHEALHNHYTQKSLSLSPGK

SEQ ID NO: 54 - DNA, 1068 bp, Artificial Sequence
  1A10-V2
caggtgcagctggtggagtccggcggcggactggtgcagcctggaggatctctgcggctgtcctgcgccgccagcggatactccagcaacgtggcttgcatggcctggtatcggcaggcccctggcaaggagcgggagtgggtgagcaccatcgtggctgacttcggcaccaccaattatgccgctagcgtgaagggccggttcaccatcagccaggataactccaagaataccgtgtatctgcagatgaatagcctgcgggccgaggataccgccgtgtattattgtgccgctacccagcggggcggcatcgactggtgtgatgagatcaactattggggccagggcaccctggtgaccgtgtcctccggcgagcctaagtcctccgacaagacccacacctgccctccttgtcccgcccctgagctgctgggcggaccatctgtgttcctgttccctcccaagcccaaggacaccctgatgatctccaggacccctgaggtgacctgcgtggtggtggatgtgtcccacgaggaccctgaggtgaagttcaactggtacgtggacggcgtggaggtgcacaatgctaagaccaagccccgggaggagcagtataacagcacctaccgggtggtgagcgtgctgaccgtgctgcaccaggattggctgaatggcaaggagtacaagtgtaaggtgtccaacaaggctctgcctgcccccatcgagaagaccatctccaaggccaagggccagcctcgggagccccaggtgtataccctgcccccctccagggacgagctgaccaagaaccaggtgagcctgacctgtctggtgaagggcttctatccttccgacatcgccgtggagtgggagtccaacggccagcctgagaataactacaagaccaccccccctgtgctggatagcgacggctccttcttcctgtattccaagctgaccgtggataagtcccggtggcagcagggcaatgtgttcagctgttccgtgatgcacgaggctctgcacaaccactatacccagaagtccctgtccctgagccccggcaag

SEQ ID NO: 55 - protein, 359 aa, Artificial Sequence
  1A11-V1
QVQLVESGGGLVQPGGSLRLSCAASGFTFNSACMGWFRQAPGKGREGVSRIETGYGGTVYADSVKGRFTISRDNSKNTVYLQMNSLRAEDTAVYYCAAKRSWCTPTWWHELDYNYWGQGTQVTVSSGEPKSSDKTHTCPPCPAPELLGGPSVFLFPPKPKDTLMISRTPEVTCVVVDVSHEDPEVKFNWYVDGVEVHNAKTKPREEQYNSTYRVVSVLTVLHQDWLNGKEYKCKVSNKALPAPIEKTISKAKGQPREPQVYTLPPSRDELTKNQVSLTCLVKGFYPSDIAVEWESNGQPENNYKTTPPVLDSDGSFFLYSKLTVDKSRWQQGNVFSCSVMHEALHNHYTQKSLSLSPGK

SEQ ID NO: 56 - DNA, 1077 bp, Artificial Sequence
  1A11-V1
caggtgcagctggtggagtccggcggcggactggtgcagccaggaggatctctgcggctgtcctgtgccgcttccggcttcaccttcaattccgcttgcatgggctggttcaggcaggcccctggcaagggcagggagggagtgtccaggatcgagaccggctacggcggcaccgtgtacgctgacagcgtgaagggccggttcaccatcagccgggataactccaagaacaccgtgtatctgcagatgaatagcctgagggctgaggataccgccgtgtactattgtgctgctaagcggtcctggtgtacccccacctggtggcacgagctggactacaattactggggccagggcacccaggtgaccgtgagctccggcgagcctaagtcctccgacaagacccacacctgccctccttgtcccgcccctgagctgctgggcggaccatctgtgttcctgttccctcccaagcccaaggacaccctgatgatctccaggacccctgaggtgacctgcgtggtggtggatgtgtcccacgaggaccctgaggtgaagttcaactggtacgtggacggcgtggaggtgcacaatgctaagaccaagccccgggaggagcagtataacagcacctaccgggtggtgagcgtgctgaccgtgctgcaccaggattggctgaatggcaaggagtacaagtgtaaggtgtccaacaaggctctgcctgcccccatcgagaagaccatctccaaggccaagggccagcctcgggagccccaggtgtataccctgcccccctccagggacgagctgaccaagaaccaggtgagcctgacctgtctggtgaagggcttctatccttccgacatcgccgtggagtgggagtccaacggccagcctgagaataactacaagaccaccccccctgtgctggatagcgacggctccttcttcctgtattccaagctgaccgtggataagtcccggtggcagcagggcaatgtgttcagctgttccgtgatgcacgaggctctgcacaaccactatacccagaagtccctgtccctgagccccggcaag

SEQ ID NO: 57 - protein, 359 aa, Artificial Sequence
  1A11-V2
QVQLVESGGGLVQPGGSLRLSCAASGFTFNSACMGWFRQAPGKEREGVSRIETGYGGTVYADSVKGRFTISRDNSKNTVYLQMNSLKAEDTAVYYCAAKRSWCTPTWWHELDYNYWGQGTQVTVSSGEPKSSDKTHTCPPCPAPELLGGPSVFLFPPKPKDTLMISRTPEVTCVVVDVSHEDPEVKFNWYVDGVEVHNAKTKPREEQYNSTYRVVSVLTVLHQDWLNGKEYKCKVSNKALPAPIEKTISKAKGQPREPQVYTLPPSRDELTKNQVSLTCLVKGFYPSDIAVEWESNGQPENNYKTTPPVLDSDGSFFLYSKLTVDKSRWQQGNVFSCSVMHEALHNHYTQKSLSLSPGK

SEQ ID NO: 58 - DNA, 1077 bp, Artificial Sequence
  1A11-V2
caggtgcagctggtggagtccggcggcggactggtgcagccaggaggatctctgcggctgtcctgtgccgcttccggcttcaccttcaattccgcttgcatgggctggttcaggcaggcccctggcaaggagagggagggagtgtccaggatcgagaccggctacggcggcaccgtgtacgctgacagcgtgaagggccggttcaccatcagccgggataactccaagaacaccgtgtatctgcagatgaatagcctgaaggctgaggataccgccgtgtactattgtgctgctaagcggtcctggtgtacccccacctggtggcacgagctggactacaattactggggccagggcacccaggtgaccgtgagctccggcgagcctaagtcctccgacaagacccacacctgccctccttgtcccgcccctgagctgctgggcggaccatctgtgttcctgttccctcccaagcccaaggacaccctgatgatctccaggacccctgaggtgacctgcgtggtggtggatgtgtcccacgaggaccctgaggtgaagttcaactggtacgtggacggcgtggaggtgcacaatgctaagaccaagccccgggaggagcagtataacagcacctaccgggtggtgagcgtgctgaccgtgctgcaccaggattggctgaatggcaaggagtacaagtgtaaggtgtccaacaaggctctgcctgcccccatcgagaagaccatctccaaggccaagggccagcctcgggagccccaggtgtataccctgcccccctccagggacgagctgaccaagaaccaggtgagcctgacctgtctggtgaagggcttctatccttccgacatcgccgtggagtgggagtccaacggccagcctgagaataactacaagaccaccccccctgtgctggatagcgacggctccttcttcctgtattccaagctgaccgtggataagtcccggtggcagcagggcaatgtgttcagctgttccgtgatgcacgaggctctgcacaaccactatacccagaagtccctgtccctgagccccggcaag

SEQ ID NO: 59 - protein, 492 aa, Artificial Sequence
  A10-linker-A11-Fc
QVQLVESGGGSVQAGGSLRLSCAASGYSSNVACMAWYRQAPGKEREWVATIVADFGTTNYAASVKGRFTISQDNAKNTVYLQMNSLKPEDSAMYYCAATQRGGIDWCDEINYWGQGTLVTVSSGGGGSGGGGSQVQLVESGGGSVQAGGSLRLSCAASGVTFNSACMGWFRQAPGKEREGVARIETGYGGTVYADSVKGRFTISRDNAKNTVYLQMNSLKPEDTAMYYCAAKRSWCTPTWWHELDYNYWGQGTQVTVSSGEPKSSDKTHTCPPCPAPEAAGGPSVFLFPPKPKDTLMISRTPEVTCVVVDVSHEDPEVKFNWYVDGVEVHNAKTKPREEQYNSTYRVVSVLTVLHQDWLNGKEYKCKVSNKALAAPIEKTISKAKGQPREPQVCTLPPSREEMTKNQVSLSCAVKGFYPSDIAVEWESNGQPENNYKTTPPVLDSDGSFFLVSKLTVDKSRWQQGNVFSCSVMHEALHNHYTQKSLSLSPGK

SEQ ID NO: 60 - DNA, 1476 bp, Artificial Sequence
  A10-linker-A11-Fc
caggtgcagctggtggagagcggcggcggatccgtgcaggctggaggaagcctgcggctgtcctgtgccgcctccggatactcctccaacgtggcctgtatggcttggtacaggcaggctcctggcaaggagcgggagtgggtggctaccatcgtggccgacttcggcaccaccaattacgctgctagcgtgaagggcaggttcaccatcagccaggataacgctaagaataccgtgtacctgcagatgaatagcctgaagcccgaggactccgctatgtactattgtgccgctacccagaggggcggcatcgattggtgcgacgagatcaattattggggccagggcaccctggtgaccgtgagcagcggcggaggcggaagcggaggaggaggaagccaggtgcagctcgtggagtccggcggcggaagcgtgcaggctggtggaagcctgaggctgtcctgtgctgctagcggcgtgaccttcaactccgcttgtatgggctggttccggcaggctcccggcaaggagagagagggcgtggccaggatcgagaccggctatggcggcaccgtgtacgccgacagcgtgaagggacggttcaccatctccagggataacgctaaaaacaccgtgtatctgcagatgaacagcctgaagccagaggataccgctatgtattactgtgctgccaagcggagctggtgtacccctacctggtggcacgagctggactacaactattggggccagggaacccaggtgaccgtgtccagcggcgagcccaagtccagcgacaagacccacacctgtcctccttgccctgctccagaggccgctggcggacctagcgtgttcctgttccctcctaagcctaaggacaccctgatgatctccagaacacctgaagtgacctgcgtggtcgtggatgtttctcacgaggaccctgaggtgaagttcaactggtacgtggacggcgtggaagtgcacaacgccaagaccaagcctcgggaggaacagtacaactccacctacagagtggtgtccgtgctgaccgtgctgcaccaggactggctgaacggaaaagagtacaagtgcaaggtgtccaacaaggccctggccgctcctatcgagaagactatctccaaggctaagggccagcctagagagcctcaagtgtgcaccctgcctccatctcgggaagagatgaccaagaaccaggtgtctctgtcttgcgccgtcaagggcttctacccttccgacatcgccgtggaatgggagtctaacggccagcctgagaacaactacaagaccacccctcctgtgctggactctgacggctccttcttcctcgtgtccaagctgaccgtggacaagtctcggtggcagcagggcaacgtgttctcctgctctgtgatgcacgaggctctgcacaaccactacacccagaagtccctgtccctgtcccctggcaag

SEQ ID NO: 61 - protein, 455 aa, Artificial Sequence
  anti-CD3-HC-Fc
EVQLVESGGGLVQPGGSLRLSCAASGFTFNTYAMNWVRQAPGKGLEWVARIRSKYNNYATYYADSVKDRFTISRDDSKNTAYLQMNNLKTEDTAMYYCVRHGNFGNSYVSWFAYWGQGTLVTVSSASTKGPSVFPLAPSSKSTSGGTAALGCLVKDYFPEPVTVSWNSGALTSGVHTFPAVLQSSGLYSLSSVVTVPSSSLGTQTYICNVNHKPSNTKVDKKVEPKSCDKTHTCPPCPAPEAAGGPSVFLFPPKPKDTLMISRTPEVTCVVVDVSHEDPEVKFNWYVDGVEVHNAKTKPREEQYNSTYRVVSVLTVLHQDWLNGKEYKCKVSNKALAAPIEKTISKAKGQPREPQVYTLPPCREEMTKNQVSLWCLVKGFYPSDIAVEWESNGQPENNYKTTPPVLDSDGSFFLYSKLTVDKSRWQQGNVFSCSVMHEALHNRFTQKSLSLSPGK

SEQ ID NO: 62 - DNA, 1365 bp, Artificial Sequence
  anti-CD3-HC-Fc
gaggtgcagctggtggaatctggcggaggcctcgtgcagcccggcggctctctgagactgtcttgcgccgcttctggctttaccttcaatacctatgccatgaattgggtgcggcaggcccctggcaagggcctggaatgggtcgccagaatcagatccaagtacaacaactacgccacctactacgccgattctgtgaaagacagattcaccatctctcgggacgactctaagaacaccgcctacctgcagatgaacaacctgaagaccgaggacaccgctatgtactactgcgtgagacacggcaacttcggcaactcctacgtgtcctggttcgcctactggggccagggcaccctggtcacagtttcttctgcctctaccaagggcccttccgtgttccctctggcccctagcagcaaaagcacctccggcggaaccgccgccctgggctgtctggtgaaggactacttccccgagcctgtgacggtgtcttggaactccggcgctctgacctctggcgtgcatacctttcctgccgtgctgcagtccagcggactgtactccctgtcctccgtcgtgacagttccctcctctagcctgggcacacagacctacatctgcaacgtgaaccacaagccttctaacaccaaagtggacaagaaggtggaacccaaatcctgcgacaagacacacacctgtcctccttgccctgctcctgaggccgctggcggccctagcgtgtttctgtttcctcctaagcccaaggacacactgatgatctccagaaccccagaagtgacctgcgtagtggtggacgtgtcccacgaggatcctgaggtgaagttcaactggtacgtggatggcgtggaagtgcacaacgccaagaccaagcctagagaagagcagtacaactccacctacagagtggtgtccgtgctgaccgtgctgcaccaggactggctgaacggcaaagagtacaagtgcaaggtgtccaacaaggccctggctgctcctatcgagaagaccatctccaaggctaagggacagcctcgggaacctcaagtgtacaccctgcctccttgtagagaggaaatgaccaagaaccaggtgtctctgtggtgcctggtcaagggcttctacccttctgacatcgccgtggagtgggagtccaacggccagcctgagaacaactacaaaaccacccctccagtgctggactccgacggctccttcttcctgtactccaagctgacagtggataagtctagatggcagcagggcaatgtgttctcctgctccgtgatgcacgaggctctgcacaaccggttcacccagaagtccctgtccctgtcccctggcaag

SEQ ID NO: 63 - protein, 215 aa, Artificial Sequence
  anti-CD3-LC
ELVVTQEPSLTTSPGGTVTLTCRSSTGAVTTSNYANWVQQKPGQAPRGLIGGTNKRAPGTPARFSGSLLGGKAALTITGVQPEDEAEYYCALWYSNLWVFGGGTKLTVLGQPKANPTVTLFPPSSEELQANKATLVCLISDFYPGAVTVAWKADGSPVKAGVETTKPSKQSNNKYAASSYLSLTPEQWKSHRSYSCQVTHEGSTVEKTVAPTECS

SEQ ID NO: 64 - DNA, 645 bp, Artificial Sequence
  anti-CD3-LC
gagctggtggtgacccaggagccatccctgaccacaagcccaggaggaaccgtgacactgacctgtagatccagcaccggcgccgtgaccacaagcaactacgctaattgggtgcagcagaagcctggacaggctccaaggggactgatcggaggaaccaacaagagagcccccggaacaccagctcggttttccggcagcctgctgggaggcaaggccgctctgacaatcaccggcgtgcagccagaggacgaggccgagtactattgcgctctgtggtattctaatctgtgggtgtttggaggaggaacaaagctgaccgtgctgggacagcccaaggctaaccctacagtgaccctgttccccccttcttccgaggagctgcaggccaataaggccaccctggtgtgcctgatctctgacttttacccaggagctgtgacagtggcttggaaggctgatggctcccctgtgaaggctggcgtggagaccacaaagccaagcaagcagtctaacaataagtacgccgctagctcttatctgtctctgacccccgagcagtggaagtcccacaggtcttattcctgccaggtgacacatgagggcagcacagtggagaagaccgtggcccctacagagtgttct

SEQ ID NO: 65 - protein, 492 aa, Artificial Sequence
  anti-BCMA-A10-v1-linker-A11-v1-Fc
QVQLVESGGGLVQPGGSLRLSCAASGYSSNVACMAWYRQAPGKGLEWVATIVADFGTTNYAASVKGRFTISQDNSKNTVYLQMNSLRAEDTAVYYCAATQRGGIDWCDEINYWGQGTLVTVSSGGGGSGGGGSQVQLVESGGGLVQPGGSLRLSCAASGFTFNSACMGWFRQAPGKGREGVSRIETGYGGTVYADSVKGRFTISRDNSKNTVYLQMNSLRAEDTAVYYCAAKRSWCTPTWWHELDYNYWGQGTQVTVSSGEPKSSDKTHTCPPCPAPEAAGGPSVFLFPPKPKDTLMISRTPEVTCVVVDVSHEDPEVKFNWYVDGVEVHNAKTKPREEQYNSTYRVVSVLTVLHQDWLNGKEYKCKVSNKALAAPIEKTISKAKGQPREPQVCTLPPSREEMTKNQVSLSCAVKGFYPSDIAVEWESNGQPENNYKTTPPVLDSDGSFFLVSKLTVDKSRWQQGNVFSCSVMHEALHNHYTQKSLSLSPGK

SEQ ID NO: 66 - DNA, 1476 bp, Artificial Sequence
  anti-BCMA-A10-v1-linker-A11-v1-Fc
caagtgcagctggtcgagtccggcggcggactggtgcagccaggcggctccctccggctgtcctgtgccgcctccggctactcctctaacgtggcctgcatggcctggtatagacaggctcctggcaagggcctggaatgggtggccaccattgtggccgacttcggcaccaccaactacgccgcttccgtcaagggcagattcaccatctcccaggataactccaagaacaccgtgtacctgcagatgaactccctgagggctgaagataccgctgtgtactactgtgctgccacacagagaggcggcatcgattggtgcgacgagatcaactattggggacagggcactttggtgaccgtgtccagcggaggcggcggctccggcgggggcggctctcaggttcagctggtcgagtccggcggtggcctggtgcagcccggcggaagcctgagactgtcctgcgccgcctctggctttaccttcaactctgcctgtatgggctggtttcggcaagcccctgggaaaggcagagagggcgtgagccggatcgagacaggctacggcggcacagtttacgctgactctgtgaagggaagattcaccatcagccgggacaattccaaaaataccgtgtacctgcagatgaacagcctgcgggccgaggacacagctgtctactactgcgcggccaagcggtcttggtgtacccctacctggtggcacgagctggactacaactactggggccagggaactcaggtgaccgtgtcctccggcgagcccaagtcctctgacaagacacacacctgtcctccatgccctgctcctgaggccgctggcggaccttccgtgttcctgtttcctcctaagcccaaggacaccctgatgatctctcggacccctgaggtgacctgcgtggtggtggacgtgtctcatgaggatcctgaagtgaagttcaactggtacgtggatggcgtggaagtgcacaacgccaagaccaagcctagagaagaacagtacaactccacctacagagtggtcagcgtgctgaccgtgctgcatcaggactggctgaacggaaaagagtacaagtgcaaggtgtccaacaaggctctggctgcccctatcgagaagaccatctccaaggccaagggccagccccgcgagcctcaggtgtgcaccctgcctccatctagagaagagatgaccaagaaccaggtctccctcagctgcgccgtgaagggcttctacccttctgacatcgctgtggaatgggaaagcaatggccaacccgagaacaactacaagaccaccccccctgtgctggactccgacggcagcttcttcctggtgtcaaagctgacagtggacaagtccagatggcagcagggcaacgtgttcagctgcagtgtgatgcacgaggccctgcacaaccactacacccagaaatctctgtctctgtctcctggcaaa

SEQ ID NO: 67 - protein, 482 aa, Artificial Sequence
  anti-CD3-scFv-Fc
ELVVTQEPSLTTSPGGTVTLTCRSSTGAVTTSNYANWVQQKPGQAPRGLIGGTNKRAPGTPARFSGSLLGGKAALTITGVQPEDEAEYYCALWYSNLWVFGGGTKLTVLGGGGSGGGGSGGGGSEVQLVESGGGLVQPGGSLRLSCAASGFTFNTYAMNWVRQAPGKGLEWVARIRSKYNNYATYYADSVKDRFTISRDDSKNTAYLQMNNLKTEDTAMYYCVRHGNFGNSYVSWFAYWGQGTLVTVSSGEPKSSDKTHTCPPCPAPEAAGGPSVFLFPPKPKDTLMISRTPEVTCVVVDVSHEDPEVKFNWYVDGVEVHNAKTKPREEQYNSTYRVVSVLTVLHQDWLNGKEYKCKVSNKALAAPIEKTISKAKGQPREPQVYTLPPCREEMTKNQVSLWCLVKGFYPSDIAVEWESNGQPENNYKTTPPVLDSDGSFFLYSKLTVDKSRWQQGNVFSCSVMHEALHNRFTQKSLSLSPGK

SEQ ID NO: 68 - DNA, 1446 bp, Artificial Sequence
  anti-CD3-scFv-Fc
gagctggtcgtcacccaagagccctctctgaccacaagccctggcggaaccgtgaccctgacctgtaggtcctccaccggcgctgtgaccacctcgaactatgccaactgggtgcaacagaagcccggccaggcacccagaggcctgatcggcggcaccaacaagcgcgcccccggcacacctgccagattctctggctctctgctgggcggaaaggccgccctgaccatcaccggcgtccagcccgaggacgaggccgagtactactgcgctctgtggtactccaacctgtgggtgtttggcggcggcaccaagctgaccgtgctgggcggcggtggctctggaggaggcggatctggtggcggaggctctgaagtgcagctcgttgagagcggcggcggcctggtgcagcctggcggctccctgagactgtcttgcgccgcttccggcttcaccttcaacacctatgccatgaattgggtccggcaggcccccggcaagggactggaatgggtggctagaatcagatccaagtacaacaactacgctacctactacgccgactctgtgaaggaccggttcaccatctctcgggacgactccaagaacaccgcctacctgcagatgaacaatctgaagaccgaggataccgctatgtactactgtgtgcggcacggcaacttcggcaactcctacgtgtcctggttcgcctactggggccagggcactctcgtgaccgtgtccagcggcgagcccaagtcctctgacaagacccacacctgccctccatgtcctgctcctgaggctgctggcggcccttccgtgtttctgttccctcctaagcctaaagatacactgatgatctcccggacccctgaagttacatgcgtggtggtggacgtgtctcacgaggaccccgaagtgaagttcaactggtatgtggatggcgtggaagtgcacaatgccaaaaccaagcctcgggaggaacagtacaactctacctacagagtggtaagcgtgctgaccgtgctgcaccaggactggctgaacggcaaagagtacaagtgcaaggtgtctaacaaggctctggccgcccctatcgagaagacaatttccaaggccaagggccagcctagagaacctcaggtgtacaccctgcctccttgcagagaagagatgaccaagaaccaggttagcctatggtgcctggtgaagggtttctacccttctgacatcgccgtggagtgggagtccaatggccaaccagagaacaactacaagacaacaccacctgtgctggactccgatggctccttcttcctgtactctaagctgacagtggacaagtccagatggcagcagggcaacgtgttctcctgctccgtgatgcatgaagctctgcacaaccggttcacccagaaatccctgagcctgtctcctggaaaa

SEQ ID NO: 69 - protein, 356 aa, Artificial Sequence
  anti-BCMA-A10-v1-Fc
QVQLVESGGGLVQPGGSLRLSCAASGYSSNVACMAWYRQAPGKGLEWVATIVADFGTTNYAASVKGRFTISQDNSKNTVYLQMNSLRAEDTAVYYCAATQRGGIDWCDEINYWGQGTLVTVSSGEPKSSDKTHTCPPCPAPEAAGGPSVFLFPPKPKDTLMISRTPEVTCVVVDVSHEDPEVKFNWYVDGVEVHNAKTKPREEQYNSTYRVVSVLTVLHQDWLNGKEYKCKVSNKALAAPIEKTISKAKGQPREPQVCTLPPSREEMTKNQVSLSCAVKGFYPSDIAVEWESNGQPENNYKTTPPVLDSDGSFFLVSKLTVDKSRWQQGNVFSCSVMHEALHNHYTQKSLSLSPGK

SEQ ID NO: 70 - DNA, 1068 bp, Artificial Sequence
  anti-BCMA-A10-v1-Fc
caagtccagctggttgagtccggcggaggcctggtgcagccaggcggctccctgagactgtcttgtgctgcctctggctactcctctaatgtggcctgcatggcctggtaccggcaggcccctggcaagggcctggaatgggtggctactatcgtggccgacttcggcaccaccaattatgctgcctctgtgaagggacggttcaccatctcccaggacaactccaagaacaccgtgtacctgcagatgaacagcctgcgggccgaggacacagccgtgtactactgtgccgctacacagagaggcggcatcgactggtgcgacgagatcaactactggggccaaggaaccctggtgacagtgtcttctggcgagcccaaatcctccgataaaacacacacctgtcctccttgccctgctcccgaggccgccggcggccctagcgtattcctgtttccccctaagcctaaggacacattgatgatctctcggacacccgaagtgacctgcgtggtcgtggacgtgtctcacgaagatcctgaggtgaagttcaactggtatgtggatggcgtggaagtgcataacgccaagaccaagcccagagaggaacagtacaactctacctacagagtggtgtccgtcctgaccgtgctgcatcaggattggctgaacggcaaagagtacaagtgcaaggtgtctaacaaggctctggccgctcccattgagaagaccatctccaaggctaagggtcagcctagagagcctcaagtgtgcaccctgcctccatctagagaagagatgaccaagaaccaggtcagcctgtcttgtgcagtgaaaggcttctacccaagcgacatcgccgtggaatgggagtctaatggccagcctgaaaacaactacaagaccacccctcctgtgctcgactccgacggctccttcttcctggtgtccaagctgaccgtggacaagtcccgctggcagcagggcaacgtgttctcctgctccgtgatgcacgaggctctgcacaaccactacacccagaagagcctgagcctgtcccctggaaag

SEQ ID NO: 71 - protein, 613 aa, Artificial Sequence
  anti-BCMA-A11-v1-linker-anti-CD3-scFv-Fc
QVQLVESGGGLVQPGGSLRLSCAASGFTFNSACMGWFRQAPGKGREGVSRIETGYGGTVYADSVKGRFTISRDNSKNTVYLQMNSLRAEDTAVYYCAAKRSWCTPTWWHELDYNYWGQGTQVTVSSGGGGSELVVTQEPSLTTSPGGTVTLTCRSSTGAVTTSNYANWVQQKPGQAPRGLIGGTNKRAPGTPARFSGSLLGGKAALTITGVQPEDEAEYYCALWYSNLWVFGGGTKLTVLGGGGSGGGGSGGGGSEVQLVESGGGLVQPGGSLRLSCAASGFTFNTYAMNWVRQAPGKGLEWVARIRSKYNNYATYYADSVKDRFTISRDDSKNTAYLQMNNLKTEDTAMYYCVRHGNFGNSYVSWFAYWGQGTLVTVSSGEPKSSDKTHTCPPCPAPEAAGGPSVFLFPPKPKDTLMISRTPEVTCVVVDVSHEDPEVKFNWYVDGVEVHNAKTKPREEQYNSTYRVVSVLTVLHQDWLNGKEYKCKVSNKALAAPIEKTISKAKGQPREPQVYTLPPCREEMTKNQVSLWCLVKGFYPSDIAVEWESNGQPENNYKTTPPVLDSDGSFFLYSKLTVDKSRWQQGNVFSCSVMHEALHNRFTQKSLSLSPGK

SEQ ID NO: 72 - DNA, 1839 bp, Artificial Sequence
  anti-BCMA-A11-v1-linker-anti-CD3-scFv-Fc
caggtgcagctcgtggaatccggcggcggcctggtgcagcctggcggctctctgagactgtcttgtgctgcctctggctttactttcaactccgcctgcatgggctggttcagacaggcccccggaaagggccgggagggcgtgtctcggatcgagacaggctacggcggtaccgtgtacgccgactctgtgaaaggcagattcaccatctccagagacaactccaagaataccgtctacctgcagatgaatagcctccgcgccgaggacaccgctgtgtactactgcgccgctaagagatcttggtgcacccccacctggtggcacgagctggactacaactactggggccagggaacccaggtgaccgtgtccagcggcggaggcggctctgaactggtggtgacccaagagccttccctgaccacctcccctggcggcacagtgacactgacctgtagatcctccaccggcgccgtgaccacctctaactatgctaactgggtgcagcagaaacctggccaggcacctcggggactgatcggcggcaccaacaagcgggctcctggaacacctgctagattctccggctccttgctgggcggcaaggccgccctgaccatcaccggggtgcaacctgaggacgaggctgagtattactgcgctctgtggtactccaacctgtgggtctttggcggcggaaccaagctgaccgtgctgggcggcggcggctccggcggaggcggctccggaggaggcggcagcgaggtgcagctggtcgagtctggcggcggcctggtgcagcccggcggctcgctgcggctgagctgtgccgcctccggcttcacattcaatacctacgccatgaactgggtcaggcaggctcctggcaaaggcctggaatgggtggccagaatccggagcaagtacaacaactatgccacctactacgccgattctgtgaaggacagattcacaatctcccgggacgactctaagaacaccgcttacctgcagatgaacaacctgaagaccgaggatacagctatgtactactgtgtgcggcacggcaacttcggcaattcctacgtgtcctggttcgcctactggggacaaggcaccttggtgacagtttctagcggcgagcccaagtcttctgacaagacacacacctgccctccttgtcctgcccctgaggccgctggcggaccttctgtgtttctgtttccacctaagcctaaggataccctgatgatctctagaacccccgaggtgacctgcgtggtcgtggacgtgagccatgaagatcctgaagtgaagttcaactggtatgtggacggcgtggaagtgcacaatgccaagaccaagcctagagaagagcagtacaactctacctacagagtggtgtccgtgctgaccgttctgcatcaggactggctgaacggcaaagagtacaagtgcaaggtgtctaacaaggctctggctgcccctatcgagaagaccatttccaaggccaagggccagccacgcgaacctcaagtgtacaccctgccaccttgcagagaggagatgaccaagaaccaggtgagcctgtggtgcctggtgaaaggcttctaccccagcgacatcgccgtggaatgggagtccaacggccagcccgagaacaactacaaaaccacccctcctgtgctggattctgatggttccttcttcctgtactctaagctgaccgtggacaagtcccggtggcagcagggcaacgtgttcagctgctccgtgatgcacgaagccctgcacaaccggttcacccagaaatccctgtctctgtctccaggcaag

SEQ ID NO: 73 - protein, 359 aa, Artificial Sequence
  anti-BCMA-A11-v1-Fc
QVQLVESGGGLVQPGGSLRLSCAASGFTFNSACMGWFRQAPGKGREGVSRIETGYGGTVYADSVKGRFTISRDNSKNTVYLQMNSLRAEDTAVYYCAAKRSWCTPTWWHELDYNYWGQGTQVTVSSGEPKSSDKTHTCPPCPAPEAAGGPSVFLFPPKPKDTLMISRTPEVTCVVVDVSHEDPEVKFNWYVDGVEVHNAKTKPREEQYNSTYRVVSVLTVLHQDWLNGKEYKCKVSNKALAAPIEKTISKAKGQPREPQVCTLPPSREEMTKNQVSLSCAVKGFYPSDIAVEWESNGQPENNYKTTPPVLDSDGSFFLVSKLTVDKSRWQQGNVFSCSVMHEALHNHYTQKSLSLSPGK

SEQ ID NO: 74 - DNA, 1077 bp, Artificial Sequence
  anti-BCMA-A11-v1-Fc
caggtgcagctggtggaatccggcggaggcctggtccagcctggaggcagcctgcggctgtcgtgcgctgcctccggattcaccttcaactccgcctgtatgggctggttcagacaggcccctggcaagggtcgcgagggcgttagccggatcgaaacaggctacggcggaaccgtctacgccgactccgtgaaaggcagattcaccatctctcgggacaattctaagaataccgtgtacctgcagatgaactctctgagggccgaggacaccgctgtgtactactgcgccgctaaacggtcctggtgcactcctacctggtggcatgagctggactacaattattggggccaaggaacacaagtgacagtatcctctggcgagcccaagtcctccgataaaacccacacctgccctccttgtcctgctccagaggccgctggcggcccttccgtgtttctgtttccacctaagcccaaggacacactgatgatcagcagaacccctgaagtcacctgtgtggtcgtggacgtgagccatgaagatcctgaggtgaagttcaactggtacgtggacggcgtggaagtgcacaacgctaaaaccaagcctagagaggaacagtacaactctacctacagagtggtgtccgtgctgacagtgctgcaccaggactggctgaacggcaaagagtacaagtgcaaggtgagtaacaaggccctggctgctcccatcgagaagaccatctccaaggccaagggccagcctcgggagcctcaggtgtgcaccctgcctccatctagagaagagatgaccaagaaccaggtgtccctgtcttgtgccgtcaagggcttctacccttctgacatcgccgtggaatgggagtctaacggccagcccgagaacaactataagaccaccccccccgtgctggattctgatggctccttcttcctcgtgtccaagctgaccgtggacaagtccagatggcagcagggcaacgtgttctcctgctctgtgatgcacgaggcactgcacaaccactacacccagaagtcccttagcctgtctcctggcaag

SEQ ID NO: 75 - protein, 343 aa, Artificial Sequence
  anti-BCMA-A10-v1-linker-anti-CD3-VL
QVQLVESGGGLVQPGGSLRLSCAASGYSSNVACMAWYRQAPGKGLEWVATIVADFGTTNYAASVKGRFTISQDNSKNTVYLQMNSLRAEDTAVYYCAATQRGGIDWCDEINYWGQGTLVTVSSGGGGSELVVTQEPSLTTSPGGTVTLTCRSSTGAVTTSNYANWVQQKPGQAPRGLIGGTNKRAPGTPARFSGSLLGGKAALTITGVQPEDEAEYYCALWYSNLWVFGGGTKLTVLGQPKANPTVTLFPPSSEELQANKATLVCLISDFYPGAVTVAWKADGSPVKAGVETTKPSKQSNNKYAASSYLSLTPEQWKSHRSYSCQVTHEGSTVEKTVAPTECS

SEQ ID NO: 76 - DNA, 1029 bp, Artificial Sequence
  anti-BCMA-A10-v1-linker-anti-CD3-VL
caagtgcagctggtggaatctggcggcggactggtgcagccaggcggctccctgagactgtcctgtgctgcttctggctactcgtccaacgtggcctgcatggcctggtatcgccaggctcctggcaaaggcctggaatgggtggctaccatcgtggccgacttcggcactacaaactacgccgcctccgtgaagggcagattcaccatctctcaggacaactccaagaacaccgtgtacctgcagatgaacagcctgcgggctgaggacaccgccgtgtactactgtgccgctacccagcggggaggcatcgactggtgcgacgagatcaactactggggccagggaaccttggttacagtgtccagcggcggaggcggctccgaactggtggtgacccaagagccttctctgaccacctcccctggcggcacagtgaccctgacctgtagatcctctaccggtgccgtgacaacctctaattacgccaactgggtccagcagaagcccggccaagcccctagaggcctgatcggcgggacgaacaagcgggctcctggcacccctgcccggttcagcggctctctgctgggcggcaaggctgccctgacaatcaccggcgtgcagcctgaggatgaggccgagtactactgcgctctgtggtatagcaacctgtgggtgttcggaggaggcacaaagctgaccgtgctgggccagcctaaggccaatcctaccgtgaccctgtttcctccatcttctgaagagctgcaggccaacaaagccaccctcgtgtgcctgatctccgacttctaccccggcgctgtgaccgtggcatggaaggccgatggctcccctgtgaaagctggcgtcgaaaccaccaagcctagcaagcagtccaacaacaagtacgctgcctcttcctacctgtctctgacccccgagcagtggaagtcccatagaagctactcttgccaggtgacccacgagggctccaccgtcgagaagaccgtggcccccaccgagtgctcc

SEQ ID NO: 77 - protein, 446 aa, Artificial Sequence
  anti-BCMA-HC-Fc
EVQLLESGGGLVQPGGSLRLSCAASGFTFSSYAMSWVRQAPGKGLEWVSAISGSGGSTYYADSVKGRFTISRDNSKNTLYLQMNSLRAEDTAVYYCAKVLGWFDYWGQGTLVTVSSASTKGPSVFPLAPSSKSTSGGTAALGCLVEDYFPEPVTVSWNSGALTSGVHTFPAVLQSSGLYSLSSVVTVPSSSLGTQTYICNVNHKPSNTKVDEKVEPKSCDKTHTCPPCPAPEAAGGPSVFLFPPKPKDTLMISRTPEVTCVVVDVSHEDPEVKFNWYVDGVEVHNAKTKPREEQYNSTYRVVSVLTVLHQDWLNGKEYKCKVSNKALGAPIEKTISKAKGQPREPQVCTLPPSRDELTKNQVSLSCAVKGFYPSDIAVEWESNGQPENNYKTTPPVLDSDGSFFLVSKLTVDKSRWQQGNVFSCSVMHEALHNRFTQKSLSLSPGK

SEQ ID NO: 78 - DNA, 1338 bp, Artificial Sequence
  anti-BCMA-HC-Fc
gaggtgcagctgctggaatctggaggcggcctggtgcaacccggcggatctctgagactgtcttgtgccgcttctggcttcaccttttcctcctacgccatgtcctgggtcagacaggcccctggaaagggactggaatgggtgtctgccatctccggctctggcggctctacatactacgccgacagcgtgaagggcagattcaccatcagccgggacaactccaagaacaccctctacctgcagatgaactctctgcgggccgaggataccgccgtgtactactgcgccaaagtgctgggatggttcgactactggggccaaggcacgctcgtgaccgtgtcctccgcctccaccaaaggaccttccgtgtttcctctggccccttccagcaagtccacctccggcggtaccgctgccctgggctgcctggtcgaggactacttccctgagcccgtgaccgtgtcttggaactccggcgctctgacctctggcgtgcacaccttccccgctgttctgcagtccagcggcctgtactccctgtcctctgtggtgacagtgcctagctcttctctgggcacccagacctacatctgcaacgtgaaccacaagccctccaacaccaaggtggatgagaaagtggaacccaagtcttgcgacaagacacatacctgtcctccttgccctgctcctgaggccgctggcggcccttctgtgttcctgttcccacccaagcctaaggacaccctgatgatctctcggacccctgaggtcacctgcgtggtcgtggacgtgtcccatgaagatcctgaagtgaagttcaactggtacgtggatggcgtggaagtgcacaacgccaagaccaagcctcgggaagagcagtacaactccacatacagagtggtgagcgtgctgaccgtgctgcaccaggactggctgaacggcaaagagtacaagtgcaaggtgtccaacaaggctctcggcgcccccatcgagaagacaatctccaaggccaagggccagcctagagagcctcaggtgtgcaccctgcctccatctcgcgacgagctgactaagaaccaggtgtccctgtcctgtgctgtgaaaggcttctacccttctgacatcgccgtggagtgggagtctaacggccagcccgagaacaactacaagaccacacctcctgttctggactccgacggctccttcttcctggtgtctaagctgaccgtggacaagtccagatggcagcagggcaacgtgttctcctgctccgtgatgcacgaggctctgcacaacagattcacccagaagtctctcagcctgtcccctggcaag

SEQ ID NO: 79 - protein, 216 aa, Artificial Sequence
  anti-BCMA-LC
EIVLTQSPGTLSLSPGERATLSCRASQSVSSSYLAWYQQKPGQAPRLLIYGASSRATGIPDRFSGSGSGTDFTLTISRLEPEDFAVYYCQQYGYPPDFTFGQGTKVEIKRTVAAPSVFIFPPSDRKLKSGTASVVCLLNNFYPREAKVQWKVDNALQSGNSQESVTEQDSKDSTYSLSSTLTLSKADYEKHKVYACEVTHQGLSSPVTKSFNRGEC

SEQ ID NO: 80 - DNA, 648 bp, Artificial Sequence
  anti-BCMA-LC
gagatcgtgctgacccagtctcctggaacactgtctctgtcccctggcgagagagctaccctgagctgcagagcctctcagtccgtgtcctcctcctacctggcctggtaccagcagaagcctggccaggcccctcggctgctgatctacggcgctagctctcgggccaccggcatccctgacagattctccggctccggctctggcacagattttaccctgaccatctccagactggaacctgaggacttcgccgtgtactactgccagcagtacggctacccccccgacttcaccttcggccaaggcaccaaagtggaaatcaagcggaccgtggctgctccttctgtgttcatcttccctccttccgaccggaagctgaagtctggaaccgcctccgtggtgtgcctgctgaacaacttctaccctagagaggccaaggtgcagtggaaggtggacaacgccctgcagagcggcaactcccaagagtccgtcaccgagcaggactctaaggactccacctactccctgtcctctaccctgacactgtccaaggccgactacgagaagcacaaggtgtacgcctgcgaggtgacccaccagggcctgtcttctcctgtgaccaagtccttcaacagaggcgaatgt

SEQ ID NO: 81 - protein, 671 aa, Artificial Sequence
  anti-BCMA-VH-anti-CD3-VL-Fc
EVQLLESGGGLVQPGGSLRLSCAASGFTFSSYAMSWVRQAPGKGLEWVSAISGSGGSTYYADSVKGRFTISRDNSKNTLYLQMNSLRAEDTAVYYCAKVLGWFDYWGQGTLVTVSSASTKGPSVFPLAPSSKSTSGGTAALGCLVEDYFPEPVTVSWNSGALTSGVHTFPAVLQSSGLYSLSSVVTVPSSSLGTQTYICNVNHKPSNTKVDEKVEPKSCDGGGGSGGGGSQAVVTQEPSLTVSPGGTVTLTCGSSTGAVTTSNYANWVQEKPGQAFRGLIGGTNKRAPGTPARFSGSLLGGKAALTLSGAQPEDEAEYYCALWYSNLWVFGGGTKLTVLSSASTKGPSVFPLAPSSKSTSGGTAALGCLVKDYFPEPVTVSWNSGALTSGVHTFPAVLQSSGLYSLSSVVTVPSSSLGTQTYICNVNHKPSNTKVDKKVEPKSCDKTHTCPPCPAPEAAGGPSVFLFPPKPKDTLMISRTPEVTCVVVDVSHEDPEVKFNWYVDGVEVHNAKTKPREEQYNSTYRVVSVLTVLHQDWLNGKEYKCKVSNKALGAPIEKTISKAKGQPREPQVYTLPPCRDELTKNQVSLWCLVKGFYPSDIAVEWESNGQPENNYKTTPPVLDSDGSFFLYSKLTVDKSRWQQGNVFSCSVMHEALHNHYTQKSLSLSPGK

SEQ ID NO: 82 - DNA, 2013 bp, Artificial Sequence
  anti-BCMA-VH-anti-CD3-VL-Fc
gaggtgcagctgctggaatcaggcggaggcctcgtgcagccaggtggcagcctgcggctgtcttgtgccgcctctggcttcaccttctcctcctacgccatgtcctgggtgcggcaggcccctggcaagggactggagtgggtctccgccatctctgggtccggaggctccacctactacgctgattctgtgaaaggcagattcaccatctctcgggacaactccaagaacacactgtacctgcagatgaactccctgagagccgaggacaccgccgtgtactactgcgccaaggtgctgggatggttcgactactggggccagggcaccttagtgaccgtgtcaagcgccagcacaaagggacctagcgtatttcctctggcccctagctctaagtccacctctggtggcaccgcagccctgggctgtctggtggaagactacttccctgaacccgtgacagtgtcttggaactccggcgctctgacatctggcgtgcacaccttccctgctgttcttcaatcttccggcctgtacagcctgtcctctgttgtcacagtgcccagttcttctctgggcacccagacatacatctgtaacgtgaaccacaagccttccaacaccaaagtggacgagaaagtggaacctaagtcctgcgatggcggcggcgggtccggtggagggggatctcaggctgtggtcacccaagagccctccctgaccgtgtcccctggcggcaccgtgacactgacctgcggctcttccacaggcgccgtgaccacctccaactacgccaactgggtgcaagagaagcctggccaggccttcagaggcctgatcggcggaaccaacaagcgggctcctggcacccctgccagattctctggaagtctgctgggtggcaaggctgcactgaccctgtccggcgctcaacctgaggatgaggccgagtactactgcgccctgtggtattccaacctgtgggtcttcggcggtggcaccaagctgaccgtgctgtcttctgcctccaccaaaggcccctcggtgttccctctggctcctagttccaagtctacctccggcggtacagctgctctgggctgcctggtcaaggattacttcccagagcctgtgaccgtgtcttggaactcgggcgccctgacttctggagtgcacacattccctgctgtgctgcagtcctctggcctgtactctctgtcttcggtcgtgacagtgccttccagcagcctcggcacacagacctacatctgcaacgtgaatcacaagcccagcaacaccaaggtggataagaaggtggaacccaaatcttgcgacaagacccacacctgtcctccttgtcctgcccctgaggccgctggcggcccttctgtgttcctgttcccgccaaagcctaaggacacgctgatgatctcccggacccctgaggtgacctgcgtggtggtggatgtgtctcatgaggaccctgaagtgaagttcaactggtacgtggacggcgtcgaggtgcacaacgccaaaaccaagcccagagaggaacagtacaacagcacctacagagtggtgtccgtgctgaccgtgctgcaccaggactggctgaacggcaaagagtacaagtgcaaggtgagcaataaggccctgggcgcccctatcgagaagaccatctccaaggccaagggccagcctagagaacctcaggtgtacaccctgcctccttgcagagacgagctgaccaagaaccaggtctctctgtggtgcctggtgaagggcttctacccttctgacatcgccgtggaatgggagtccaatggacagcccgagaacaactacaagaccacacctccagtgctggactccgacggctccttcttcctgtacagcaagctgacagtggacaagtccagatggcagcagggcaacgtgttctcctgctccgtgatgcacgaggctctgcacaaccactacacccagaagtccctgtccctgtctcctggaaag

SEQ ID NO: 83 - protein, 232 aa, Artificial Sequence
  anti-CD3-VH-CL
EVQLLESGGGLVQPGGSLRLSCAASGFTFSTYAMNWVRQAPGKGLEWVSRIRSKYNNYATYYADSVKGRFTISRDDSKNTLYLQMNSLRAEDTAVYYCVRHGNFGNSYVSWFAYWGQGTLVTVSSASVAAPSVFIFPPSDEQLKSGTASVVCLLNNFYPREAKVQWKVDNALQSGNSQESVTEQDSKDSTYSLSSTLTLSKADYEKHKVYACEVTHQGLSSPVTKSFNRGEC

SEQ ID NO: 84 - DNA, 696 bp, Artificial Sequence
  anti-CD3-VH-CL
gaggtgcagctgctggaatccggcggaggactggtccagcctggcggctctctgcggctgtcttgtgctgcttctggcttcaccttctccacatatgccatgaactgggtcagacaggcccccggcaagggcctggaatgggtgtccagaatcagatccaagtacaacaactacgccacctactacgccgattccgtgaagggacggttcaccatctcccgggacgactccaagaacacactgtacctgcagatgaacagcctgagagccgaggacaccgccgtgtactactgcgtgcggcacggcaacttcggcaattcctacgtgtcctggttcgcctactggggccagggcaccctggtcaccgtgtcttccgcctctgtggccgctccttctgtgttcatcttccctccttccgacgagcagctgaagtctggcacagcttctgtggtgtgcctgctgaacaacttctaccctagagaggccaaggtgcagtggaaggtggacaacgccctgcagtccggcaactcccaagagtccgtgaccgagcaggactctaaggactctacctactccctgtcctccaccctgaccctgagcaaggccgactacgagaagcacaaagtgtacgcctgcgaagtgacccaccagggcctgtcctctcctgtgaccaagtccttcaacagaggcgagtgc